European Patent Specification EP 2 953 978 B1, published October 23, 2024. Title: PHOSPHORYLCHOLINE CONJUGATES AND USES THEREOF. Applicant: TEL HASHOMER MEDICAL RESEARCH INFRASTRUCTURE AND SERVICES LTD. The sequence listing filed with the application follows.

SEQUENCE LISTING (22 sequences)

SEQ ID NO: 1 - DNA, 16 bp, Artificial Sequence
  IFN-gamma primer
gaacgctacacactgc

SEQ ID NO: 2 - DNA, 16 bp, Artificial Sequence
  IFN-gamma primer
ctggacctgtgggttg

SEQ ID NO: 3 - DNA, 17 bp, Artificial Sequence
  IL-1beta primer
ccccaactggtaaatca

SEQ ID NO: 4 - DNA, 17 bp, Artificial Sequence
  IL-1beta primer
ccgaggactaaggagtg

SEQ ID NO: 5 - DNA, 18 bp, Artificial Sequence
  IL-10 primer
aacctcgtttgtacctct

SEQ ID NO: 6 - DNA, 16 bp, Artificial Sequence
  IL-10 primer
caccatagcaaagggc

SEQ ID NO: 7 - DNA, 20 bp, Artificial Sequence
  IL-17a primer
gggcaagggatgctctctag

SEQ ID NO: 8 - DNA, 20 bp, Artificial Sequence
  IL-17a primer
ctgaagctgctgcagagctg

SEQ ID NO: 9 - DNA, 17 bp, Artificial Sequence
  TNF-alpha primer
acgtcgtagcaaaccac

SEQ ID NO: 10 - DNA, 17 bp, Artificial Sequence
  TNF-alpha primer
agatagcaaatcggctg

SEQ ID NO: 11 - DNA, 16 bp, Artificial Sequence
  TGF-beta primer
gaacccccattgctgt

SEQ ID NO: 12 - DNA, 16 bp, Artificial Sequence
  TGF-beta primer
gccctgtattccgtct

SEQ ID NO: 13 - DNA, 18 bp, Artificial Sequence
  Foxp3 primer
taccacaatatgcgaccc

SEQ ID NO: 14 - DNA, 20 bp, Artificial Sequence
  Foxp3 primer
ctcaaattcatctacggtcc

SEQ ID NO: 15 - DNA, 16 bp, beta-actin
gtgacgttgacatccg

SEQ ID NO: 16 - DNA, 16 bp, Artificial Sequence
  beta-actin primer
cagtaacagtccgcct

SEQ ID NO: 17 - protein, 4 aa, Artificial Sequence
  synthetic peptide
TKPR

SEQ ID NO: 18 - protein, 4 aa, Artificial Sequence
  synthetic peptide
  MISC_FEATURE (4)..(4): X is abcent or Arg.
  MISC_FEATURE (4)..(4): X is absent or Arg.
TKPX

SEQ ID NO: 19 - protein, 5 aa, Artificial Sequence
  synthetic peptide
TKPPR

SEQ ID NO: 20 - protein, 4 aa, Artificial Sequence
  synthetic peptide
SKPR

SEQ ID NO: 21 - protein, 4 aa, Artificial Sequence
  synthetic peptide
TRPR

SEQ ID NO: 22 - protein, 4 aa, Artificial Sequence
  synthetic peptide
SKPK